European Patent Specification EP 3 516 072 B1, published May 6, 2026. Title: METHOD FOR QUANTIFYING AND/OR DETECTING HUMAN MALE DNA. Applicant: Qiagen GmbH. The sequence listing filed with the application follows.

SEQUENCE LISTING (45 sequences)

SEQ ID NO: 1 - DNA, 22 bp, Artificial Sequence
  Synthetic Primer
gaaaggcctcatcagggctcag

SEQ ID NO: 2 - DNA, 27 bp, Artificial Sequence
  Synthetic Primer
tcctcactgggaaacatgaggaatgac

SEQ ID NO: 3 - DNA, 81 bp, Homo sapiens
gaaaggcctcatcagggctcagaaaggtgacccaagcagctgggaacacacggggtcattcctcatgtttcccagtgagga

SEQ ID NO: 4 - DNA, 81 bp, Homo sapiens; identical to SEQ ID NO: 3

SEQ ID NO: 5 - DNA, 81 bp, Homo sapiens
gaaaggcctcatcagggctcagaaaggtgacccaagcagctgggaacacatggggtcattcctcatgtttcccagtgagga

SEQ ID NO: 6 - DNA, 81 bp, Homo sapiens; identical to SEQ ID NO: 3

SEQ ID NO: 7 - DNA, 81 bp, Homo sapiens; identical to SEQ ID NO: 3

SEQ ID NO: 8 - DNA, 81 bp, Homo sapiens; identical to SEQ ID NO: 3

SEQ ID NO: 9 - DNA, 81 bp, Homo sapiens; identical to SEQ ID NO: 3

SEQ ID NO: 10 - DNA, 81 bp, Homo sapiens; identical to SEQ ID NO: 5

SEQ ID NO: 11 - DNA, 81 bp, Homo sapiens; identical to SEQ ID NO: 3

SEQ ID NO: 12 - DNA, 25 bp, Artificial Sequence
  Synthetic Probe
ggtgacccaagcagctgggaacaca

SEQ ID NO: 13 - DNA, 26 bp, Artificial Sequence
  Synthetic Primer
catgaacgtcctggattctgtcactc

SEQ ID NO: 14 - DNA, 33 bp, Artificial Sequence
  Synthetic Primer
tcactctctgtcttcctctcaaggaatttctac

SEQ ID NO: 15 - DNA, 26 bp, Artificial Sequence
  Synthetic Primer
gccatgaacgtcctggattctgtcac

SEQ ID NO: 16 - DNA, 25 bp, Artificial Sequence
  Synthetic Probe
caggctccctgaataggcaggtgtg

SEQ ID NO: 17 - DNA, 359 bp, Homo sapiens
tcctcactgggaaacatgaggaatgaccccgtgtgttcccagctgcttgggtcacctttctgagccctgatgaggcctttcccgattgagtcccctgacagatcctatgtaaggacctgtggcgcaatcccctgcaatactacaagaggatgaagccacctgaagagggaacagagacgtcaggtgagccgttagttggcactggagctgtttgatgcccagtataagggggttgacacacctgcctattcagggagcctgggtgctcatttcagaaatgtagaaattgaggctcctttcgtacatgtagaaattccttgagaggaagacagagagtgacagaatccaggacgttcatg

SEQ ID NO: 18 - DNA, 359 bp, Homo sapiens; identical to SEQ ID NO: 17

SEQ ID NO: 19 - DNA, 359 bp, Homo sapiens
tcctcactgggaaacatgaggaatgaccccatgtgttcccagctgcttgggtcacctttctgagccctgatgaggcctttcccgattgagtcccctgacagatcctatgtaaggacctgtggcgcaatcccctgcaatactacaagaggatgaagccacctgaagagggaacagagacgtcaggtgagccgttagttggcactggagctgtttgatgcccagtataagggggttgacacacctgcctattcagggagcctgggtgctcatttcagaaatgtagaaattgaggctcctttcgtacatgtagaaattccttgagaggaagacagagagtgacagaatccaggacgttcatg

SEQ ID NO: 20 - DNA, 357 bp, Homo sapiens
tcctcactgggaaacatgaggaatgaccccgtgtgttcccagctgcttgggtcacctttctgagccctgatgaggcctttcccgattgagtcccctgacagatcctatgtaaggacctgtggcgcaatcccctgcaatactacaagaggatgaagccacctgaagagggaacagagacgtcaggtgagccgttagttggcactggagctgtttgatgcgcagtataagggggttgacacacctgcctattcagggagcctgggtgctcatttcagaaatgtagaaactgaggctcctttcgtacatgtagaaattccttgagaggaagacagagtgacagaatccaggacgttcatg

SEQ ID NO: 21 - DNA, 359 bp, Homo sapiens; identical to SEQ ID NO: 17

SEQ ID NO: 22 - DNA, 359 bp, Homo sapiens; identical to SEQ ID NO: 17

SEQ ID NO: 23 - DNA, 359 bp, Homo sapiens; identical to SEQ ID NO: 17

SEQ ID NO: 24 - DNA, 359 bp, Homo sapiens; identical to SEQ ID NO: 19

SEQ ID NO: 25 - DNA, 359 bp, Homo sapiens; identical to SEQ ID NO: 17

SEQ ID NO: 26 - DNA, 340 bp, Homo sapiens
tcctcactgggaaacatgaggaatgaccccatgtgttcccagctgcttgggtcaccattctgagtcctgatgaggcctttcccgatggattcccctgacagatcctatgtaaggacctgtggtgcaatcccctgcaatcctacaagaggatgaagccacctgaagagggaacagagatttcaggtgagctgttcagttggaactgaagctttttgatccccaggataaggaggttgacacacctgcctattcagggagcctggaggctcatttcagaaatgtagaaattgagcctcctttcatacatgtagaaattccttgagaggaagacagagtgtga

SEQ ID NO: 27 - DNA, 339 bp, Homo sapiens
tcctcactgggaaacatgaggaatgaccccgtgtgttcccagctgcttgggtcacctttctgagccctgatgaggcctttcccgattgagtcccctgacagatcctatgtaaggacctgtggcgcaatcccctgcaatactacaagaggatgaagccacctgaagagggaacagagacgtcaggtgagccgttagttggcactggagctgtttgatgcccagtataagggggttgacacacctgcctattcagggagcctgggtgctcatttcagaaatgtagaaattgaggctcctttcgtacatgtagaaattccttgagaggaagacagagagtga

SEQ ID NO: 28 - DNA, 339 bp, Homo sapiens; identical to SEQ ID NO: 27

SEQ ID NO: 29 - DNA, 339 bp, Homo sapiens
tcctcactgggaaacatgaggaatgaccccatgtgttcccagctgcttgggtcacctttctgagccctgatgaggcctttcccgattgagtcccctgacagatcctatgtaaggacctgtggcgcaatcccctgcaatactacaagaggatgaagccacctgaagagggaacagagacgtcaggtgagccgttagttggcactggagctgtttgatgcccagtataagggggttgacacacctgcctattcagggagcctgggtgctcatttcagaaatgtagaaattgaggctcctttcgtacatgtagaaattccttgagaggaagacagagagtga

SEQ ID NO: 30 - DNA, 339 bp, Homo sapiens
tcctcactgggaaacatgaggaatgaccccgtgtgttcccagctgcttgggtcacctttctgagccctgatgaggcctttcccgattgagtcccctgacagatcctatgtaaggacctgtggcgcaatcccctgcaatactacaagaggatgaagccacctgaagagggaacagagacgtcaggtgagccgttagttggcactggagctgtttgatgcgcagtataagggggttgacacacctgcctattcagggagcctgggtgctcatttcagaaatgtagaaactgaggctcctttcgtacatgtagaaattccttgagaggaagacagagtgaca

SEQ ID NO: 31 - DNA, 339 bp, Homo sapiens; identical to SEQ ID NO: 27

SEQ ID NO: 32 - DNA, 339 bp, Homo sapiens; identical to SEQ ID NO: 27

SEQ ID NO: 33 - DNA, 339 bp, Homo sapiens; identical to SEQ ID NO: 27

SEQ ID NO: 34 - DNA, 339 bp, Homo sapiens; identical to SEQ ID NO: 29

SEQ ID NO: 35 - DNA, 339 bp, Homo sapiens; identical to SEQ ID NO: 27

SEQ ID NO: 36 - DNA, 362 bp, Homo sapiens
tcctcactgggaaacatgaggaatgaccccatgtgttcccagctgcttgggtcaccattctgagtcctgatgaggcctttcccgatggattcccctgacagatcctatgtaaggacctgtggtgcaatcccctgcaatcctacaagaggatgaagccacctgaagagggaacagagatttcaggtgagctgttcagttggaactgaagctttttgatccccaggataaggaggttgacacacctgcctattcagggagcctggaggctcatttcagaaatgtagaaattgagcctcctttcatacatgtagaaattccttgagaggaagacagagtgtgacagaatccaggacattcatggc

SEQ ID NO: 37 - DNA, 361 bp, Homo sapiens
tcctcactgggaaacatgaggaatgaccccgtgtgttcccagctgcttgggtcacctttctgagccctgatgaggcctttcccgattgagtcccctgacagatcctatgtaaggacctgtggcgcaatcccctgcaatactacaagaggatgaagccacctgaagagggaacagagacgtcaggtgagccgttagttggcactggagctgtttgatgcccagtataagggggttgacacacctgcctattcagggagcctgggtgctcatttcagaaatgtagaaattgaggctcctttcgtacatgtagaaattccttgagaggaagacagagagtgacagaatccaggacgttcatggc

SEQ ID NO: 38 - DNA, 361 bp, Homo sapiens; identical to SEQ ID NO: 37

SEQ ID NO: 39 - DNA, 361 bp, Homo sapiens
tcctcactgggaaacatgaggaatgaccccatgtgttcccagctgcttgggtcacctttctgagccctgatgaggcctttcccgattgagtcccctgacagatcctatgtaaggacctgtggcgcaatcccctgcaatactacaagaggatgaagccacctgaagagggaacagagacgtcaggtgagccgttagttggcactggagctgtttgatgcccagtataagggggttgacacacctgcctattcagggagcctgggtgctcatttcagaaatgtagaaattgaggctcctttcgtacatgtagaaattccttgagaggaagacagagagtgacagaatccaggacgttcatggc

SEQ ID NO: 40 - DNA, 359 bp, Homo sapiens
tcctcactgggaaacatgaggaatgaccccgtgtgttcccagctgcttgggtcacctttctgagccctgatgaggcctttcccgattgagtcccctgacagatcctatgtaaggacctgtggcgcaatcccctgcaatactacaagaggatgaagccacctgaagagggaacagagacgtcaggtgagccgttagttggcactggagctgtttgatgcgcagtataagggggttgacacacctgcctattcagggagcctgggtgctcatttcagaaatgtagaaactgaggctcctttcgtacatgtagaaattccttgagaggaagacagagtgacagaatccaggacgttcatggc

SEQ ID NO: 41 - DNA, 361 bp, Homo sapiens; identical to SEQ ID NO: 37

SEQ ID NO: 42 - DNA, 361 bp, Homo sapiens; identical to SEQ ID NO: 37

SEQ ID NO: 43 - DNA, 361 bp, Homo sapiens; identical to SEQ ID NO: 37

SEQ ID NO: 44 - DNA, 361 bp, Homo sapiens; identical to SEQ ID NO: 39

SEQ ID NO: 45 - DNA, 361 bp, Homo sapiens; identical to SEQ ID NO: 37